European Patent Application EP 4 570 816 A1, published June 18, 2025. Title: Soluble gp130Fc (sgp130Fc) for the treatment of SARS-CoV-2. Applicant: Consejo Superior de Investigaciones Cientificas (CSIC). The sequence listing filed with the application follows.

SEQUENCE LISTING (48 sequences)

SEQ ID NO: 1 - protein, 822 aa, synthetic construct
  source 1..822: note = amino acid sequence of the Interleukin-6 trans-signaling inhibitor, fusion protein sgp130Fc; note (original language) = secuencia de aminoacidos del inihibidor de la transeñalizacion de la interleukina 6, proteina de fusion sgp130Fc; organism (original language) = construccion sintetica
ELLDPCGYISPESPVVQLHSNFTAVCVLKEKCMDYFHVNANYIVWKTNHFTIPKEQYTIINRTASSVTFTDIASLNIQLTCNILTFGQLEQNVYGITIISGLPPEKPKNLSCIVNEGKKMRCEWDGGRETHLETNFTLKSEWATHKFADCKAKRDTPTSCTVDYSTVYFVNIEVWVEAENALGKVTSDHINFDPVYKVKPNPPHNLSVINSEELSSILKLTWTNPSIKSVIILKYNIQYRTKDASTWSQIPPEDTASTRSSFTVQDLKPFTEYVFRIRCMKEDGKGYWSDWSEEASGITYEDRPSKAPSFWYKIDPSHTQGYRTVQLVWKTLPPFEANGKILDYEVTLTRWKSHLQNYTVNATKLTVNLTNDRYLATLTVRNLVGKSDAAVLTIPACDFQATHPVMDLKAFPKDNMLWVEWTTPRESVKKYILEWCVLSDKAPCITDWQQEDGTVHRTYLRGNLAESKCYLITVTPVYADGPGSPESIKAYLKQAPPSKGPTVRTKKVGKNEAVLEWDQLPVDVQNGFIRNYTIFYRTIIGNETAVNVDSSHTEYTLSSLTSDTLYMVRMAAYTDEGGKDGPEFTFTTPKFAQGEDKTHTCPPCPAPEAEGAPSVFLFPPKPKDTLMISRTPEVTCVVVDVSHEDPEVKFNWYVDGVEVHNAKTKPREEQYNSTYRVVSVLTVLHQDWLNGKEYKCKVSNKALPAPIEKTISKAKGQPREPQVYTLPPSREEMTKNQVSLTCLVKGFYPSDIAVEWESNGQPENNYKTTPPVLDSDGSFFLYSKLTVDKSRWQQGNVFSCSVMHEALHNHYTQKSLSLSPGK

SEQ ID NO: 2 - DNA, 20 bp, synthetic construct
  source 1..20: mol_type = other DNA; note = primer; note (original language) = cebador; organism (original language) = construccion sintetica
gtctccttcgagctgtttgc

SEQ ID NO: 3 - DNA, 20 bp, synthetic construct
  source 1..20: mol_type = other DNA; note = primer; note (original language) = cebador; organism (original language) = construccion sintetica
cgtgtaaagtcaccaccctg

SEQ ID NO: 4 - DNA, 18 bp, synthetic construct
  source 1..18: mol_type = other DNA; note = primer; note (original language) = cebador; organism (original language) = construccion sintetica
acgaaggctgtgctttgc

SEQ ID NO: 5 - DNA, 20 bp, synthetic construct
  source 1..20: mol_type = other DNA; note = primer; note (original language) = cebador; organism (original language) = construccion sintetica
ttcgttgtggctggacttgc

SEQ ID NO: 6 - DNA, 20 bp, synthetic construct
  source 1..20: mol_type = other DNA; note = primer; note (original language) = cebador; organism (original language) = construccion sintetica
acggcttctaagaacactgc

SEQ ID NO: 7 - DNA, 20 bp, synthetic construct
  source 1..20: mol_type = other DNA; note = primer; note (original language) = cebador; organism (original language) = construccion sintetica
gatatagggctccaagagtg

SEQ ID NO: 8 - DNA, 21 bp, synthetic construct
  source 1..21: mol_type = other DNA; note = primer; note (original language) = cebador; organism (original language) = construccion sintetica
cgagaccacgctccagtatat

SEQ ID NO: 9 - DNA, 21 bp, synthetic construct
  source 1..21: mol_type = other DNA; note = primer; note (original language) = cebador; organism (original language) = construccion sintetica
tttccagtgcagaaccagcag

SEQ ID NO: 10 - DNA, 20 bp, synthetic construct
  source 1..20: mol_type = other DNA; note = primer; note (original language) = cebador; organism (original language) = construccion sintetica
actagctgcacagatgagag

SEQ ID NO: 11 - DNA, 20 bp, synthetic construct
  source 1..20: mol_type = other DNA; note = primer; note (original language) = cebador; organism (original language) = construccion sintetica
gctccagagtctttagggaa

SEQ ID NO: 12 - DNA, 18 bp, synthetic construct
  source 1..18: mol_type = other DNA; note = primer; note (original language) = cebador; organism (original language) = construccion sintetica
aaggccggagatttcgct

SEQ ID NO: 13 - DNA, 20 bp, synthetic construct
  source 1..20: mol_type = other DNA; note = primer; note (original language) = cebador; organism (original language) = construccion sintetica
aacttgctgtgggtgaccat

SEQ ID NO: 14 - DNA, 22 bp, synthetic construct
  source 1..22: mol_type = other DNA; note = primer; note (original language) = cebador; organism (original language) = construccion sintetica
tagaggagcagctatggtctct

SEQ ID NO: 15 - DNA, 22 bp, synthetic construct
  source 1..22: mol_type = other DNA; note = primer; note (original language) = cebador; organism (original language) = construccion sintetica
taccctcagccgactgcagtat

SEQ ID NO: 16 - DNA, 21 bp, synthetic construct
  source 1..21: mol_type = other DNA; note = primer; note (original language) = cebador; organism (original language) = construccion sintetica
cttgggatccacactctccag

SEQ ID NO: 17 - DNA, 20 bp, synthetic construct
  source 1..20: mol_type = other DNA; note = primer; note (original language) = cebador; organism (original language) = construccion sintetica
aaatacctgtggccttgggc

SEQ ID NO: 18 - DNA, 21 bp, synthetic construct
  source 1..21: mol_type = other DNA; note = primer; note (original language) = cebador; organism (original language) = construccion sintetica
agacaaggtcccaaagacagc

SEQ ID NO: 19 - DNA, 21 bp, synthetic construct
  source 1..21: mol_type = other DNA; note = primer; note (original language) = cebador; organism (original language) = construccion sintetica
cagtgccattatggcgtgtga

SEQ ID NO: 20 - DNA, 20 bp, synthetic construct
  source 1..20: mol_type = other DNA; note = primer; note (original language) = cebador; organism (original language) = construccion sintetica
ttgacgttgcagacttggct

SEQ ID NO: 21 - DNA, 20 bp, synthetic construct
  source 1..20: mol_type = other DNA; note = primer; note (original language) = cebador; organism (original language) = construccion sintetica
aactggagattcaggactga

SEQ ID NO: 22 - DNA, 21 bp, synthetic construct
  source 1..21: mol_type = other DNA; note = primer; note (original language) = cebador; organism (original language) = construccion sintetica
gcagaaagcttgtctcaaccc

SEQ ID NO: 23 - DNA, 22 bp, synthetic construct
  source 1..22: mol_type = other DNA; note = primer; note (original language) = cebador; organism (original language) = construccion sintetica
ggcagaaagcttgtctcaaccc

SEQ ID NO: 24 - DNA, 20 bp, synthetic construct
  source 1..20: mol_type = other DNA; note = primer; note (original language) = cebador; organism (original language) = construccion sintetica
aacatctcccccttctcctt

SEQ ID NO: 25 - DNA, 20 bp, synthetic construct
  source 1..20: mol_type = other DNA; note = primer; note (original language) = cebador; organism (original language) = construccion sintetica
gaaggccttgaccttttcag

SEQ ID NO: 26 - DNA, 21 bp, synthetic construct
  source 1..21: mol_type = other DNA; note = primer; note (original language) = cebador; organism (original language) = construccion sintetica
aaggatttggctagcgcaagc

SEQ ID NO: 27 - DNA, 21 bp, synthetic construct
  source 1..21: mol_type = other DNA; note = primer; note (original language) = cebador; organism (original language) = construccion sintetica
ccacacgatgtagctggcatt

SEQ ID NO: 28 - DNA, 21 bp, synthetic construct
  source 1..21: mol_type = other DNA; note = primer; note (original language) = cebador; organism (original language) = construccion sintetica
tcttggaggagcctttaccat

SEQ ID NO: 29 - DNA, 20 bp, synthetic construct
  source 1..20: mol_type = other DNA; note = primer; note (original language) = cebador; organism (original language) = construccion sintetica
tttccaggaactccagttgc

SEQ ID NO: 30 - DNA, 21 bp, synthetic construct
  source 1..21: mol_type = other DNA; note = primer; note (original language) = cebador; organism (original language) = construccion sintetica
cgatgcatgcaaacggtctga

SEQ ID NO: 31 - DNA, 21 bp, synthetic construct
  source 1..21: mol_type = other DNA; note = primer; note (original language) = cebador; organism (original language) = construccion sintetica
gacttcgtgatcaccaggtga

SEQ ID NO: 32 - DNA, 20 bp, synthetic construct
  source 1..20: mol_type = other DNA; note = primer; note (original language) = cebador; organism (original language) = construccion sintetica
cctggagacatctgtcctca

SEQ ID NO: 33 - DNA, 20 bp, synthetic construct
  source 1..20: mol_type = other DNA; note = primer; note (original language) = cebador; organism (original language) = construccion sintetica
cctgagcagctgctgctcat

SEQ ID NO: 34 - DNA, 18 bp, synthetic construct
  source 1..18: mol_type = other DNA; note = primer; note (original language) = cebador; organism (original language) = construccion sintetica
ttgttcacgaggctttcc

SEQ ID NO: 35 - DNA, 19 bp, synthetic construct
  source 1..19: mol_type = other DNA; note = primer; note (original language) = cebador; organism (original language) = construccion sintetica
tgagcagcatcatagttcc

SEQ ID NO: 36 - DNA, 20 bp, synthetic construct
  source 1..20: mol_type = other DNA; note = primer; note (original language) = cebador; organism (original language) = construccion sintetica
agcccacgtcgtagcaaacc

SEQ ID NO: 37 - DNA, 20 bp, synthetic construct
  source 1..20: mol_type = other DNA; note = primer; note (original language) = cebador; organism (original language) = construccion sintetica
gaggagcacgtagtcggggc

SEQ ID NO: 38 - DNA, 19 bp, synthetic construct
  source 1..19: mol_type = other DNA; note = primer; note (original language) = cebador; organism (original language) = construccion sintetica
acagcaaggcgaaaaagga

SEQ ID NO: 39 - DNA, 19 bp, synthetic construct
  source 1..19: mol_type = other DNA; note = primer; note (original language) = cebador; organism (original language) = construccion sintetica
tggtggaccactcggatga

SEQ ID NO: 40 - DNA, 18 bp, synthetic construct
  source 1..18: mol_type = other DNA; note = primer; note (original language) = cebador; organism (original language) = construccion sintetica
tgacccaaccacaaatgc

SEQ ID NO: 41 - DNA, 20 bp, synthetic construct
  source 1..20: mol_type = other DNA; note = primer; note (original language) = cebador; organism (original language) = construccion sintetica
ctggctctgaaacaaaggat

SEQ ID NO: 42 - DNA, 20 bp, synthetic construct
  source 1..20: mol_type = other DNA; note = primer; note (original language) = cebador; organism (original language) = construccion sintetica
gcaagtgtcccaaagaagct

SEQ ID NO: 43 - DNA, 20 bp, synthetic construct
  source 1..20: mol_type = other DNA; note = primer; note (original language) = cebador; organism (original language) = construccion sintetica
agcttctttgggacacttgc

SEQ ID NO: 44 - DNA, 20 bp, synthetic construct
  source 1..20: mol_type = other DNA; note = primer; note (original language) = cebador; organism (original language) = construccion sintetica
aggatggcactttcccactg

SEQ ID NO: 45 - DNA, 20 bp, synthetic construct
  source 1..20: mol_type = other DNA; note = primer; note (original language) = cebador; organism (original language) = construccion sintetica
ggagagcacattcacggtca

SEQ ID NO: 46 - protein, 95 aa, synthetic construct
  source 1..95: note = a fragment of the extracellular region of gp130; note (original language) = un fragmento de la region extracelular de gp130; organism (original language) = Construccion sintetica
ELLDPCGYISPESPVVQLHSNFTAVCVLKEKCMDYFHVNANYIVWKTNHFTIPKEQYTIINRTASSVTFTDIASLNIQLTCNILTFGQLEQNVYG

SEQ ID NO: 47 - protein, 595 aa, synthetic construct
  source 1..595: note = a fragment of the extracellular region of gp130; note (original language) = un fragmento de la region extracelular de gp130; organism (original language) = construccion sintetica
ELLDPCGYISPESPVVQLHSNFTAVCVLKEKCMDYFHVNANYIVWKTNHFTIPKEQYTIINRTASSVTFTDIASLNIQLTCNILTFGQLEQNVYGITIISGLPPEKPKNLSCIVNEGKKMRCEWDGGRETHLETNFTLKSEWATHKFADCKAKRDTPTSCTVDYSTVYFVNIEVWVEAENALGKVTSDHINFDPVYKVKPNPPHNLSVINSEELSSILKLTWTNPSIKSVIILKYNIQYRTKDASTWSQIPPEDTASTRSSFTVQDLKPFTEYVFRIRCMKEDGKGYWSDWSEEASGITYEDRPSKAPSFWYKIDPSHTQGYRTVQLVWKTLPPFEANGKILDYEVTLTRWKSHLQNYTVNATKLTVNLTNDRYLATLTVRNLVGKSDAAVLTIPACDFQATHPVMDLKAFPKDNMLWVEWTTPRESVKKYILEWCVLSDKAPCITDWQQEDGTVHRTYLRGNLAESKCYLITVTPVYADGPGSPESIKAYLKQAPPSKGPTVRTKKVGKNEAVLEWDQLPVDVQNGFIRNYTIFYRTIIGNETAVNVDSSHTEYTLSSLTSDTLYMVRMAAYTDEGGKDGPEFTFTTPKFAQGE

SEQ ID NO: 48 - protein, 227 aa, synthetic construct
  source 1..227: note = constant Fc portion of IgG1; note (original language) = porcion Fc constante de IgG1; organism (original language) = construccion sintetica
DKTHTCPPCPAPEAEGAPSVFLFPPKPKDTLMISRTPEVTCVVVDVSHEDPEVKFNWYVDGVEVHNAKTKPREEQYNSTYRVVSVLTVLHQDWLNGKEYKCKVSNKALPAPIEKTISKAKGQPREPQVYTLPPSREEMTKNQVSLTCLVKGFYPSDIAVEWESNGQPENNYKTTPPVLDSDGSFFLYSKLTVDKSRWQQGNVFSCSVMHEALHNHYTQKSLSLSPGK